European Patent Specification EP 3 789 396 B1, published May 29, 2024. Title: Synthetic Peptide sp2 and Application Thereof. Applicant: Taian City Qihang Biotechnology Co. Application 18939564.3. The sequence listing filed with the application follows.

SEQUENCE LISTING (1 sequence)

SEQ ID NO: 1 - protein, 15 aa, synthesized
RVLNGPEEEAAAPAE